European Patent Specification EP 3 995 582 B1, published April 22, 2026. Title: Anti-EphA4 antibody. Applicant: EISAI R&D MANAGEMENT CO., LTD. The sequence listing filed with the application follows.

SEQUENCE LISTING (62 sequences)

SEQ ID NO: 1 - protein, 986 aa, Mus musculus
MAGIFYFILFSFLFGICDAVTGSRVYPANEVTLLDSRSVQGELGWIASPLEGGWEEVSIMDEKNTPIRTYQVCNVMEASQNNWLRTDWITREGAQRVYIEIKFTLRDCNSLPGVMGTCKETFNLYYYESDNDKERFIRESQFGKIDTIAADESFTQVDIGDRIMKLNTEIRDVGPLSKKGFYLAFQDVGACIALVSVRVFYKKCPLTVRNLAQFPDTITGADTSSLVEVRGSCVNNSEEKDVPKMYCGADGEWLVPIGNCLCNAGHEEQNGECQACKIGYYKALSTDASCAKCPPHSYSVWEGATSCTCDRGFFRADNDAASMPCTRPPSAPLNLISNVNETSVNLEWSSPQNTGGRQDISYNVVCKKCGAGDPSKCRPCGSGVHYTPQQNGLKTTRVSITDLLAHTNYTFEIWAVNGVSKYNPSPDQSVSVTVTTNQAAPSSIALVQAKEVTRYSVALAWLEPDRPNGVILEYEVKYYEKDQNERSYRIVRTAARNTDIKGLNPLTSYVFHVRARTAAGYGDFSEPLEVTTNTVPSRIIGDGANSTVLLVSVSGSVVLVVILIAAFVISRRRSKYSKAKQEADEEKHLNQGVRTYVDPFTYEDPNQAVREFAKEIDASCIKIEKVIGVGEFGEVCSGRLKVPGKREICVAIKTLKAGYTDKQRRDFLSEASIMGQFDHPNIIHLEGVVTKCKPVMIITEYMENGSLDAFLRKNDGRFTVIQLVGMLRGIGSGMKYLSDMSYVHRDLAARNILVNSNLVCKVSDFGMSRVLEDDPEAAYTTRGGKIPIRWTAPEAIAYRKFTSASDVWSYGIVMWEVMSYGERPYWDMSNQDVIKAIEEGYRLPPPMDCPIALHQLMLDCWQKERSDRPKFGQIVNMLDKLIRNPNSLKRTGSESSRPNTALLDPSSPEFSAVVSVGDWLQAIKMDRYKDNFTAAGYTTLEAVVHMSQDDLARIGITAITHQNKILSSVQAMRTQMQQMHGRMVPV

SEQ ID NO: 2 - protein, 528 aa, Mus musculus
VTGSRVYPANEVTLLDSRSVQGELGWIASPLEGGWEEVSIMDEKNTPIRTYQVCNVMEASQNNWLRTDWITREGAQRVYIEIKFTLRDCNSLPGVMGTCKETFNLYYYESDNDKERFIRESQFGKIDTIAADESFTQVDIGDRIMKLNTEIRDVGPLSKKGFYLAFQDVGACIALVSVRVFYKKCPLTVRNLAQFPDTITGADTSSLVEVRGSCVNNSEEKDVPKMYCGADGEWLVPIGNCLCNAGHEEQNGECQACKIGYYKALSTDASCAKCPPHSYSVWEGATSCTCDRGFFRADNDAASMPCTRPPSAPLNLISNVNETSVNLEWSSPQNTGGRQDISYNVVCKKCGAGDPSKCRPCGSGVHYTPQQNGLKTTRVSITDLLAHTNYTFEIWAVNGVSKYNPSPDQSVSVTVTTNQAAPSSIALVQAKEVTRYSVALAWLEPDRPNGVILEYEVKYYEKDQNERSYRIVRTAARNTDIKGLNPLTSYVFHVRARTAAGYGDFSEPLEVTTNTVPSRIIGDGANST

SEQ ID NO: 3 - protein, 1030 aa, Artificial Sequence
  Synthetic polypeptide
VTGSRVYPANEVTLLDSRSVQGELGWIASPLEGGWEEVSIMDEKNTPIRTYQVCNVMEASQNNWLRTDWITREGAQRVYIEIKFTLRDCNSLPGVMGTCKETFNLYYYESDNDKERFIRESQFGKIDTIAADESFTQVDIGDRIMKLNTEIRDVGPLSKKGFYLAFQDVGACIALVSVRVFYKKCPLTVRNLAQFPDTITGADTSSLVEVRGSCVNNSEEKDVPKMYCGADGEWLVPIGNCLCNAGHEEQNGECQACKIGYYKALSTDASCAKCPPHSYSVWEGATSCTCDRGFFRADNDAASMPCTRPPSAPLNLISNVNETSVNLEWSSPQNTGGRQDISYNVVCKKCGAGDPSKCRPCGSGVHYTPQQNGLKTTRVSITDLLAHTNYTFEIWAVNGVSKYNPSPDQSVSVTVTTNQAAPSSIALVQAKEVTRYSVALAWLEPDRPNGVILEYEVKYYEKDQNERSYRIVRTAARNTDIKGLNPLTSYVFHVRARTAAGYGDFSEPLEVTTNTVPSRIIGDGANSTAAAIIPVEEENPDFWNREAAEALGAAKKLQPAQTAAKNLIIFLGDGMGVSTVTAARILKGQKKDKLGPEIPLAMDRFPYVALSKTYNVDKHVPDSGATATAYLCGVKGNFQTIGLSAAARFNQCNTTRGNEVISVMNRAKKAGKSVGVVTTTRVQHASPAGTYAHTVNRNWYSDADVPASARQEGCQDIATQLISNMDIDVILGGGRKYMFRMGTPDPEYPDDYSQGGTRLDGKNLVQEWLAKRQGARYVWNRTELMQASLDPSVTHLMGLFEPGDMKYEIHRDSTLDPSLMEMTEAALRLLSRNPRGFFLFVEGGRIDHGHHESRAYRALTETIMFDDAIERAGQLTSEEDTLSLVTADHSHVFSFGGYPLRGSSIFGLAPGKARDRKAYTVLLYGNGPGYVLKDGARPDVTESESGSPEYRQQSAVPLDEETHAGEDVAVFARGPQAHLVHGVQEQTFIAHVMAFAACLEPYTACDLAPPAGTTDAAHPGHHHHHHHHHH

SEQ ID NO: 4 - protein, 19 aa, Mus musculus
MAGIFYFILFSFLFGICDA

SEQ ID NO: 5 - protein, 986 aa, Homo sapiens
MAGIFYFALFSCLFGICDAVTGSRVYPANEVTLLDSRSVQGELGWIASPLEGGWEEVSIMDEKNTPIRTYQVCNVMEPSQNNWLRTDWITREGAQRVYIEIKFTLRDCNSLPGVMGTCKETFNLYYYESDNDKERFIRENQFVKIDTIAADESFTQVDIGDRIMKLNTEIRDVGPLSKKGFYLAFQDVGACIALVSVRVFYKKCPLTVRNLAQFPDTITGADTSSLVEVRGSCVNNSEEKDVPKMYCGADGEWLVPIGNCLCNAGHEERSGECQACKIGYYKALSTDATCAKCPPHSYSVWEGATSCTCDRGFFRADNDAASMPCTRPPSAPLNLISNVNETSVNLEWSSPQNTGGRQDISYNVVCKKCGAGDPSKCRPCGSGVHYTPQQNGLKTTKVSITDLLAHTNYTFEIWAVNGVSKYNPNPDQSVSVTVTTNQAAPSSIALVQAKEVTRYSVALAWLEPDRPNGVILEYEVKYYEKDQNERSYRIVRTAARNTDIKGLNPLTSYVFHVRARTAAGYGDFSEPLEVTTNTVPSRIIGDGANSTVLLVSVSGSVVLVVILIAAFVISRRRSKYSKAKQEADEEKHLNQGVRTYVDPFTYEDPNQAVREFAKEIDASCIKIEKVIGVGEFGEVCSGRLKVPGKREICVAIKTLKAGYTDKQRRDFLSEASIMGQFDHPNIIHLEGVVTKCKPVMIITEYMENGSLDAFLRKNDGRFTVIQLVGMLRGIGSGMKYLSDMSYVHRDLAARNILVNSNLVCKVSDFGMSRVLEDDPEAAYTTRGGKIPIRWTAPEAIAYRKFTSASDVWSYGIVMWEVMSYGERPYWDMSNQDVIKAIEEGYRLPPPMDCPIALHQLMLDCWQKERSDRPKFGQIVNMLDKLIRNPNSLKRTGTESSRPNTALLDPSSPEFSAVVSVGDWLQAIKMDRYKDNFTAAGYTTLEAVVHVNQEDLARIGITAITHQNKILSSVQAMRTQMQQMHGRMVPV

SEQ ID NO: 6 - protein, 528 aa, Homo sapiens
VTGSRVYPANEVTLLDSRSVQGELGWIASPLEGGWEEVSIMDEKNTPIRTYQVCNVMEPSQNNWLRTDWITREGAQRVYIEIKFTLRDCNSLPGVMGTCKETFNLYYYESDNDKERFIRENQFVKIDTIAADESFTQVDIGDRIMKLNTEIRDVGPLSKKGFYLAFQDVGACIALVSVRVFYKKCPLTVRNLAQFPDTITGADTSSLVEVRGSCVNNSEEKDVPKMYCGADGEWLVPIGNCLCNAGHEERSGECQACKIGYYKALSTDATCAKCPPHSYSVWEGATSCTCDRGFFRADNDAASMPCTRPPSAPLNLISNVNETSVNLEWSSPQNTGGRQDISYNVVCKKCGAGDPSKCRPCGSGVHYTPQQNGLKTTKVSITDLLAHTNYTFEIWAVNGVSKYNPNPDQSVSVTVTTNQAAPSSIALVQAKEVTRYSVALAWLEPDRPNGVILEYEVKYYEKDQNERSYRIVRTAARNTDIKGLNPLTSYVFHVRARTAAGYGDFSEPLEVTTNTVPSRIIGDGANST

SEQ ID NO: 7 - DNA, 12 bp, Artificial Sequence
  ad29S
acatcactccgt

SEQ ID NO: 8 - DNA, 50 bp, Artificial Sequence
  ad29AS
acggagtgatgtccgtcgacgtatctctgcgttgatacttcagcgtagct

SEQ ID NO: 9 - DNA, 26 bp, Artificial Sequence
  Synthetic primer
agctacgctgaagtatcaacgcagag

SEQ ID NO: 10 - DNA, 20 bp, Artificial Sequence
  Synthetic primer
gccagtggatagactgatgg

SEQ ID NO: 11 - DNA, 21 bp, Artificial Sequence
  Synthetic primer
gatggatacagttggtgcagc

SEQ ID NO: 12 - protein, 19 aa, Artificial Sequence
  Synthetic polypeptide
MAVLVLLLCLVTFPSCVLS

SEQ ID NO: 13 - protein, 125 aa, Artificial Sequence
  Synthetic polypeptide
QVQLKQSGPSLVQPSQSLSITCTVSGFSLTRYGVHWVRQSPGKGLEWLGVIWRGGSTDYNAAFMSRLSITKDNSKSQVFFKMNSLQADDTAIYYCAKESLFGVYYDYGYYSMDYWGQGTSVTVSS

SEQ ID NO: 14 - protein, 22 aa, Artificial Sequence
  Synthetic polypeptide
MDMRVPAHVFGFLLLWFPGTRC

SEQ ID NO: 15 - protein, 107 aa, Artificial Sequence
  Synthetic polypeptide
DIQMTQSPSSLSASLGERVSLTCRASQEISGYLSWLQQKPDGTIKRLIYAASTLDSGVPKRFSGSRSGSDYSLTISSLESEDFADYYCLQYASYPLTFGAGTKLELK

SEQ ID NO: 16 - DNA, 57 bp, Artificial Sequence
  Synthetic polynucleotide
atggctgtcctggtgctgctcctctgcctggtgacattcccaagctgtgtcctgtcc

SEQ ID NO: 17 - DNA, 375 bp, Artificial Sequence
  Synthetic polynucleotide
caggtgcagctgaagcagtcaggacctagcctagtgcagccctcacagagcctgtccataacctgcacagtctctggtttctcattaactaggtatggtgtacactgggttcgccagtctccaggaaagggtctggagtggctgggagtgatttggagaggtggaagcacagactacaatgcagctttcatgtccagactgagcatcaccaaggacaactccaagagccaagttttctttaaaatgaacagtctgcaagctgatgacactgccatatactactgtgccaaagaaagcctatttggggtctactatgattacgggtactattctatggactactggggtcaaggaacctcagtcaccgtctcctca

SEQ ID NO: 18 - DNA, 66 bp, Artificial Sequence
  Synthetic polynucleotide
atggacatgagggttcctgctcacgtttttggcttcttgttgctctggtttccaggtaccagatgt

SEQ ID NO: 19 - DNA, 321 bp, Artificial Sequence
  Synthetic polynucleotide
gacatccaaatgacccagtctccatcctccttatctgcctctctgggagaaagagtcagtctcacttgtcgggcaagtcaggaaattagtggttacttaagctggcttcagcagaaaccagatggaactattaaacgcctgatctacgccgcatccactttagattctggtgtcccaaaaaggttcagtggcagtaggtctgggtcagattattctctcaccatcagcagccttgagtctgaagattttgcagactattactgtctacaatatgctagttatccgctcacgttcggtgctgggaccaagctggagctgaaa

SEQ ID NO: 20 - DNA, 40 bp, Artificial Sequence
  Synthetic primer
gcgaagcttgccgccaccatggctgtcctggtgctgctcc

SEQ ID NO: 21 - DNA, 43 bp, Artificial Sequence
  Synthetic primer
gcgaagcttgccgccaccatggacatgagggttcctgctcacg

SEQ ID NO: 22 - DNA, 36 bp, Artificial Sequence
  Synthetic primer
gcggaattcatcatttaccaggagagtgggagaggc

SEQ ID NO: 23 - DNA, 40 bp, Artificial Sequence
  Synthetic primer
cgcgaattcactaacactcattcctgttgaagctcttgac

SEQ ID NO: 24 - protein, 324 aa, Artificial Sequence
  Synthetic polypeptide
AKTTPPSVYPLAPGSAAQTNSMVTLGCLVKGYFPEPVTVTWNSGSLSSGVHTFPAVLQSDLYTLSSSVTVPSSTWPSETVTCNVAHPASSTKVDKKIVPRDCGCKPCICTVPEVSSVFIFPPKPKDVLTITLTPKVTCVVVDISKDDPEVQFSWFVDDVEVHTAQTQPREEQFNSTFRSVSELPIMHQDWLNGKEFKCRVNSAAFPAPIEKTISKTKGRPKAPQVYTIPPPKEQMAKDKVSLTCMITDFFPEDITVEWQWNGQPAENYKNTQPIMDTDGSYFVYSKLNVQKSNWEAGNTFTCSVLHEGLHNHHTEKSLSHSPGK

SEQ ID NO: 25 - protein, 107 aa, Artificial Sequence
  Synthetic polypeptide
RADAAPTVSIFPPSSEQLTSGGASVVCFLNNFYPKDINVKWKIDGSERQNGVLNSWTDQDSKDSTYSMSSTLTLTKDEYERHNSYTCEATHKTSTSPIVKSFNRNEC

SEQ ID NO: 26 - protein, 5 aa, Artificial Sequence
  Synthetic peptide
RYGVH

SEQ ID NO: 27 - protein, 16 aa, Artificial Sequence
  Synthetic peptide
VIWRGGSTDYNAAFMS

SEQ ID NO: 28 - protein, 17 aa, Artificial Sequence
  Synthetic peptide
ESLFGVYYDYGYYSMDY

SEQ ID NO: 29 - protein, 11 aa, Artificial Sequence
  Synthetic peptide
RASQEISGYLS

SEQ ID NO: 30 - protein, 7 aa, Artificial Sequence
  Synthetic peptide
AASTLDS

SEQ ID NO: 31 - protein, 9 aa, Artificial Sequence
  Synthetic peptide
LQYASYPLT

SEQ ID NO: 32 - protein, 986 aa, Macaca mulatta
MAGIFYFALFSCLFGICDAVTGSRVYPANEVTLLDSRSVQGELGWIASPLEGGWEEVSIMDEKNTPIRTYQVCNVMEPSQNNWLRTDWITREGAQRVYIEIKFTLRDCNSLPGVMGTCKETFNLYYYESDNDKERFIRENQFVKIDTIAADESFTQVDIGDRIMKLNTEIRDVGPLSKKGFYLAFQDVGACIALVSVRVFYKKCPLTVRNLAQFPDTITGADTSSLVEVRGSCVNNSEEKDVPKMYCGADGEWLVPIGNCLCNAGHEERSGECQACKIGYYKALSTDATCAKCPPHSYSVWEGATSCTCDRGFFRADNDAASMPCTRPPSAPLNLISNVNETSVNLEWSSPQNTGGRQDISYNVVCKKCGAGDPSKCRPCGSGVHYTPQQNGLKTTKVSITDLLAHTNYTFEIWAVNGVSKYNPSPDQSVSVTVTTNQAAPSSIALVQAKEVTRYSVALAWLEPDRPNGVILEYEVKYYEKDQNERSYRIVRTAARNTDIKGLNPLTSYVFHVRARTAAGYGDFSEPLEVTTNTVPSRIIGDGANSTVLLVSVSGSVVLVVILIAAFVISRRRSKYSKAKQEADEEKHLNQGVRTYVDPFTYEDPNQAVREFAKEIDASCIKIEKVIGVGEFGEVCSGRLKVPGKREICVAIKTLKAGYTDKQRRDFLSEASIMGQFDHPNIIHLEGVVTKCKPVMIITEYMENGSLDAFLRKNDGRFTVIQLVGMLRGIGSGMKYLSDMSYVHRDLAARNILVNSNLVCKVSDFGMSRVLEDDPEAAYTTRGGKIPIRWTAPEAIAYRKFTSASDVWSYGIVMWEVMSYGERPYWDMSNQDVIKAIEEGYRLPPPMDCPIALHQLMLDCWQKERSDRPKFGQIVNMLDKLIRNPNSLKRTGTESSRPNTALLDPSSPEFSAVVSVGDWLQAIKMDRYKDNFTAAGYTTLEAVVHVNQEDLARIGITAITHQNKILSSVQAMRTQMQQMHGRMVPV

SEQ ID NO: 33 - protein, 528 aa, Macaca mulatta
VTGSRVYPANEVTLLDSRSVQGELGWIASPLEGGWEEVSIMDEKNTPIRTYQVCNVMEPSQNNWLRTDWITREGAQRVYIEIKFTLRDCNSLPGVMGTCKETFNLYYYESDNDKERFIRENQFVKIDTIAADESFTQVDIGDRIMKLNTEIRDVGPLSKKGFYLAFQDVGACIALVSVRVFYKKCPLTVRNLAQFPDTITGADTSSLVEVRGSCVNNSEEKDVPKMYCGADGEWLVPIGNCLCNAGHEERSGECQACKIGYYKALSTDATCAKCPPHSYSVWEGATSCTCDRGFFRADNDAASMPCTRPPSAPLNLISNVNETSVNLEWSSPQNTGGRQDISYNVVCKKCGAGDPSKCRPCGSGVHYTPQQNGLKTTKVSITDLLAHTNYTFEIWAVNGVSKYNPSPDQSVSVTVTTNQAAPSSIALVQAKEVTRYSVALAWLEPDRPNGVILEYEVKYYEKDQNERSYRIVRTAARNTDIKGLNPLTSYVFHVRARTAAGYGDFSEPLEVTTNTVPSRIIGDGANST

SEQ ID NO: 34 - protein, 19 aa, Homo sapiens
MAGIFYFALFSCLFGICDA

SEQ ID NO: 35 - protein, 15 aa, Homo sapiens
MSALLILALVGAAVA

SEQ ID NO: 36 - protein, 547 aa, Homo sapiens
MAGIFYFALFSCLFGICDAVTGSRVYPANEVTLLDSRSVQGELGWIASPLEGGWEEVSIMDEKNTPIRTYQVCNVMEPSQNNWLRTDWITREGAQRVYIEIKFTLRDCNSLPGVMGTCKETFNLYYYESDNDKERFIRENQFVKIDTIAADESFTQVDIGDRIMKLNTEIRDVGPLSKKGFYLAFQDVGACIALVSVRVFYKKCPLTVRNLAQFPDTITGADTSSLVEVRGSCVNNSEEKDVPKMYCGADGEWLVPIGNCLCNAGHEERSGECQACKIGYYKALSTDATCAKCPPHSYSVWEGATSCTCDRGFFRADNDAASMPCTRPPSAPLNLISNVNETSVNLEWSSPQNTGGRQDISYNVVCKKCGAGDPSKCRPCGSGVHYTPQQNGLKTTKVSITDLLAHTNYTFEIWAVNGVSKYNPNPDQSVSVTVTTNQAAPSSIALVQAKEVTRYSVALAWLEPDRPNGVILEYEVKYYEKDQNERSYRIVRTAARNTDIKGLNPLTSYVFHVRARTAAGYGDFSEPLEVTTNTVPSRIIGDGANST

SEQ ID NO: 37 - protein, 328 aa, Homo sapiens
MAGIFYFALFSCLFGICDAVTGSRVYPANEVTLLDSRSVQGELGWIASPLEGGWEEVSIMDEKNTPIRTYQVCNVMEPSQNNWLRTDWITREGAQRVYIEIKFTLRDCNSLPGVMGTCKETFNLYYYESDNDKERFIRENQFVKIDTIAADESFTQVDIGDRIMKLNTEIRDVGPLSKKGFYLAFQDVGACIALVSVRVFYKKCPLTVRNLAQFPDTITGADTSSLVEVRGSCVNNSEEKDVPKMYCGADGEWLVPIGNCLCNAGHEERSGECQACKIGYYKALSTDATCAKCPPHSYSVWEGATSCTCDRGFFRADNDAASMPCTRP

SEQ ID NO: 38 - protein, 236 aa, Homo sapiens
PLTVRNLAQFPDTITGADTSSLVEVRGSCVNNSEEKDVPKMYCGADGEWLVPIGNCLCNAGHEERSGECQACKIGYYKALSTDATCAKCPPHSYSVWEGATSCTCDRGFFRADNDAASMPCTRPPSAPLNLISNVNETSVNLEWSSPQNTGGRQDISYNVVCKKCGAGDPSKCRPCGSGVHYTPQQNGLKTTKVSITDLLAHTNYTFEIWAVNGVSKYNPNPDQSVSVTVTTNQAA

SEQ ID NO: 39 - protein, 112 aa, Homo sapiens
TNQAAPSSIALVQAKEVTRYSVALAWLEPDRPNGVILEYEVKYYEKDQNERSYRIVRTAARNTDIKGLNPLTSYVFHVRARTAAGYGDFSEPLEVTTNTVPSRIIGDGANST

SEQ ID NO: 40 - protein, 96 aa, Artificial Sequence
  Synthetic polypeptide
DIQMTQSPSSLSASVGDRVTITCRASQGIRNDLGWYQQKPGKAPKRLIYAASSLQSGVPSRFSGSGSGTEFTLTISSLQPEDFATYYCLQHNSYPP

SEQ ID NO: 41 - protein, 12 aa, Artificial Sequence
  Synthetic polypeptide
LTFGGGTKVEIK

SEQ ID NO: 42 - protein, 98 aa, Artificial Sequence
  Synthetic polypeptide
QVQLVESGGGVVQPGRSLRLSCAASGFTFSSYGMHWVRQAPGKGLEWVAVIWYDGSNKYYADSVKGRFTISRDNSKNTLYLQMNSLRAEDTAVYYCAK

SEQ ID NO: 43 - protein, 18 aa, Artificial Sequence
  Synthetic polypeptide
YYYYGMDVWGQGTTVTVS

SEQ ID NO: 44 - protein, 5 aa, Artificial Sequence
  Synthetic polypeptide
RFGVH

SEQ ID NO: 45 - protein, 125 aa, Artificial Sequence
  Synthetic polypeptide
QVQLVESGGGVVQPGRSLRLSCAVSGFSLTRFGVHWVRQAPGKGLEWVAVIWRGGSTDYNAAFMSRLTISKDNSKNTVYLQMNSLRAEDTAVYYCAKESLFGVYYDYGYYSMDYWGQGTTVTVSS

SEQ ID NO: 46 - protein, 107 aa, Artificial Sequence
  Synthetic polypeptide
DIQMTQSPSSLSASVGDRVTITCRASQEISGYLSWLQQKPGKAPKRLIYAASTLDSGVPSRFSGSRSGTEYTLTISSLQPEDFATYYCLQYASYPLTFGGGTKVEIK

SEQ ID NO: 47 - protein, 326 aa, Homo sapiens
ASTKGPSVFPLAPSSRSTSESTAALGCLVKDYFPEPVTVSWNSGALTSGVHTFPAVLQSSGLYSLSSVVTVPSSNFGTQTYTCNVDHKPSNTKVDKTVERKSCVECPPCPAPPAAAPSVFLFPPKPKDTLMISRTPEVTCVVVDVSHEDPEVQFNWYVDGVEVHNAKTKPREEQFNSTFRVVSVLTVVHQDWLNGKEYKCKVSNKGLPAPIEKTISKTKGQPREPQVYTLPPSREEMTKNQVSLTCLVKGFYPSDIAVEWESNGQPENNYKTTPPMLDSDGSFFLYSKLTVDKSRWQQGNVFSCSVMHEALHNHYTQKSLSLSPGK

SEQ ID NO: 48 - protein, 107 aa, Homo sapiens [sequence omitted]

SEQ ID NO: 49 - DNA, 15 bp, Artificial Sequence
  Synthetic polynucleotide
agatttggagtgcat

SEQ ID NO: 50 - DNA, 48 bp, Artificial Sequence
  Synthetic polynucleotide
gtgatctggaggggaggatccaccgactacaacgctgcttttatgagc

SEQ ID NO: 51 - DNA, 51 bp, Artificial Sequence
  Synthetic polynucleotide
gagagcctgttcggcgtgtactatgactacggctactattctatggattat

SEQ ID NO: 52 - DNA, 33 bp, Artificial Sequence
  Synthetic polynucleotide
cgcgcctcccaggagatctctggctacctgtcc

SEQ ID NO: 53 - DNA, 21 bp, Artificial Sequence
  Synthetic polynucleotide
gctgcctccaccctggactct

SEQ ID NO: 54 - DNA, 27 bp, Artificial Sequence
  Synthetic polynucleotide
ctgcagtacgcttcctatccactgacc

SEQ ID NO: 55 - DNA, 375 bp, Artificial Sequence
  Synthetic polynucleotide
caggtgcagctggtggagagcggaggaggagtggtgcagcctggcaggtccctgaggctgagctgtgccgtgtccggcttcagcctgacaagatttggagtgcattgggtgcgccaggctccaggcaagggactggagtgggtggccgtgatctggaggggaggatccaccgactacaacgctgcttttatgagccggctgacaatctctaaggataactccaagaataccgtgtatctgcagatgaactccctgagggctgaggacaccgccgtgtactattgcgccaaggagagcctgttcggcgtgtactatgactacggctactattctatggattattggggccagggcaccacagtgacagtgtcctcc

SEQ ID NO: 56 - DNA, 321 bp, Artificial Sequence
  Synthetic polynucleotide
gatatccagatgacacagtccccttccagcctgtctgcctccgtgggcgacagagtgaccatcacatgtcgcgcctcccaggagatctctggctacctgtcctggctgcagcagaagccaggcaaggctcccaagcgcctgatctatgctgcctccaccctggactctggagtgccttccaggttcagcggctctcggtccggcacagagtacaccctgacaatctcttccctgcagcctgaggatttcgccacctactattgcctgcagtacgcttcctatccactgacctttggcggcggcacaaaggtggagatcaag

SEQ ID NO: 57 - DNA, 978 bp, Artificial Sequence
  Synthetic polynucleotide
gcctccaccaagggaccatccgtgttcccactggccccatcttcccggagcacatctgagtccaccgccgctctgggctgtctggtgaaggattacttccctgagccagtgacagtgtcttggaactccggcgctctgacatccggcgtgcacacctttcctgccgtgctgcagagctctggcctgtacagcctgtccagcgtggtgaccgtgccctcttccaatttcggcacccagacatatacctgcaacgtggaccataagccttccaatacaaaggtggataagaccgtggagagaaagagctgcgtggagtgtccaccttgcccagctccaccagccgctgcccctagcgtgttcctgtttcctccaaagccaaaggacacactgatgatctctcgcacacccgaggtgacctgcgtggtggtggacgtgtcccacgaggatccagaggtgcagtttaactggtacgtggatggcgtggaggtgcataatgctaagaccaagcccagggaggagcagttcaactccacatttcgggtggtgagcgtgctgaccgtggtgcaccaggactggctgaacggcaaggagtataagtgtaaggtgagcaataagggcctgcccgcccctatcgagaagacaatctctaagaccaagggccagcctagagagccacaggtgtacaccctgcccccttctcgcgaggagatgacaaagaaccaggtgtccctgacctgcctggtgaagggcttctatcctagcgacatcgctgtggagtgggagtctaatggccagccagagaacaattacaagaccacaccacccatgctggacagcgatggctctttctttctgtattctaagctgacagtggataagtccaggtggcagcagggcaacgtgtttagctgctctgtgatgcatgaggccctgcacaatcattacacccagaagtccctgagcctgtctccaggcaag

SEQ ID NO: 58 - DNA, 321 bp, Artificial Sequence
  Synthetic polynucleotide
aggacagtggccgctccatccgtgttcatctttccccctagcgacgagcagctgaagagcggcaccgcctctgtggtgtgcctgctgaacaatttctaccccagggaggccaaggtgcagtggaaggtggataacgctctgcagagcggcaattctcaggagtccgtgaccgagcaggacagcaaggattctacatattccctgagctctaccctgacactgagcaaggccgattacgagaagcacaaggtgtatgcttgcgaggtgacccatcagggcctgtccagcccagtgacaaagtcttttaacaggggcgagtgt

SEQ ID NO: 59 - protein, 451 aa, Artificial Sequence
  Synthetic polypeptide
QVQLVESGGGVVQPGRSLRLSCAVSGFSLTRFGVHWVRQAPGKGLEWVAVIWRGGSTDYNAAFMSRLTISKDNSKNTVYLQMNSLRAEDTAVYYCAKESLFGVYYDYGYYSMDYWGQGTTVTVSSASTKGPSVFPLAPSSRSTSESTAALGCLVKDYFPEPVTVSWNSGALTSGVHTFPAVLQSSGLYSLSSVVTVPSSNFGTQTYTCNVDHKPSNTKVDKTVERKSCVECPPCPAPPAAAPSVFLFPPKPKDTLMISRTPEVTCVVVDVSHEDPEVQFNWYVDGVEVHNAKTKPREEQFNSTFRVVSVLTVVHQDWLNGKEYKCKVSNKGLPAPIEKTISKTKGQPREPQVYTLPPSREEMTKNQVSLTCLVKGFYPSDIAVEWESNGQPENNYKTTPPMLDSDGSFFLYSKLTVDKSRWQQGNVFSCSVMHEALHNHYTQKSLSLSPGK

SEQ ID NO: 60 - protein, 214 aa, Artificial Sequence
  Synthetic polypeptide
DIQMTQSPSSLSASVGDRVTITCRASQEISGYLSWLQQKPGKAPKRLIYAASTLDSGVPSRFSGSRSGTEYTLTISSLQPEDFATYYCLQYASYPLTFGGGTKVEIKRTVAAPSVFIFPPSDEQLKSGTASVVCLLNNFYPREAKVQWKVDNALQSGNSQESVTEQDSKDSTYSLSSTLTLSKADYEKHKVYACEVTHQGLSSPVTKSFNRGEC

SEQ ID NO: 61 - DNA, 1353 bp, Artificial Sequence
  Synthetic polynucleotide
caggtgcagctggtggagagcggaggaggagtggtgcagcctggcaggtccctgaggctgagctgtgccgtgtccggcttcagcctgacaagatttggagtgcattgggtgcgccaggctccaggcaagggactggagtgggtggccgtgatctggaggggaggatccaccgactacaacgctgcttttatgagccggctgacaatctctaaggataactccaagaataccgtgtatctgcagatgaactccctgagggctgaggacaccgccgtgtactattgcgccaaggagagcctgttcggcgtgtactatgactacggctactattctatggattattggggccagggcaccacagtgacagtgtcctccgcctccaccaagggaccatccgtgttcccactggccccatcttcccggagcacatctgagtccaccgccgctctgggctgtctggtgaaggattacttccctgagccagtgacagtgtcttggaactccggcgctctgacatccggcgtgcacacctttcctgccgtgctgcagagctctggcctgtacagcctgtccagcgtggtgaccgtgccctcttccaatttcggcacccagacatatacctgcaacgtggaccataagccttccaatacaaaggtggataagaccgtggagagaaagagctgcgtggagtgtccaccttgcccagctccaccagccgctgcccctagcgtgttcctgtttcctccaaagccaaaggacacactgatgatctctcgcacacccgaggtgacctgcgtggtggtggacgtgtcccacgaggatccagaggtgcagtttaactggtacgtggatggcgtggaggtgcataatgctaagaccaagcccagggaggagcagttcaactccacatttcgggtggtgagcgtgctgaccgtggtgcaccaggactggctgaacggcaaggagtataagtgtaaggtgagcaataagggcctgcccgcccctatcgagaagacaatctctaagaccaagggccagcctagagagccacaggtgtacaccctgcccccttctcgcgaggagatgacaaagaaccaggtgtccctgacctgcctggtgaagggcttctatcctagcgacatcgctgtggagtgggagtctaatggccagccagagaacaattacaagaccacaccacccatgctggacagcgatggctctttctttctgtattctaagctgacagtggataagtccaggtggcagcagggcaacgtgtttagctgctctgtgatgcatgaggccctgcacaatcattacacccagaagtccctgagcctgtctccaggcaag

SEQ ID NO: 62 - DNA, 642 bp, Artificial Sequence
  Synthetic polynucleotide
gatatccagatgacacagtccccttccagcctgtctgcctccgtgggcgacagagtgaccatcacatgtcgcgcctcccaggagatctctggctacctgtcctggctgcagcagaagccaggcaaggctcccaagcgcctgatctatgctgcctccaccctggactctggagtgccttccaggttcagcggctctcggtccggcacagagtacaccctgacaatctcttccctgcagcctgaggatttcgccacctactattgcctgcagtacgcttcctatccactgacctttggcggcggcacaaaggtggagatcaagaggacagtggccgctccatccgtgttcatctttccccctagcgacgagcagctgaagagcggcaccgcctctgtggtgtgcctgctgaacaatttctaccccagggaggccaaggtgcagtggaaggtggataacgctctgcagagcggcaattctcaggagtccgtgaccgagcaggacagcaaggattctacatattccctgagctctaccctgacactgagcaaggccgattacgagaagcacaaggtgtatgcttgcgaggtgacccatcagggcctgtccagcccagtgacaaagtcttttaacaggggcgagtgt